European Patent Application EP 4 306 540 A1, published January 17, 2024. Title: ROR1 BINDING PROTEIN AND USE THEREOF. Applicant: SICHUAN KELUN-BIOTECH BIOPHARMACEUTICAL CO., LTD. KLUS PHARMA INC. The sequence listing filed with the application follows.

SEQUENCE LISTING (161 sequences)

SEQ ID NO: 1 - protein, 121 aa, Artificial sequence
  Murine antibody 3D8.2.3 heavy chain variable region
EVKLVESGGGLVKPGGSLKLSCAASGFTFSSYAMSWVRQTPEKRLEWVASINSGGSTYYPDSVKGRFTISRDNARNILYLQMSSLRSEDTAMYYCARVNYYGYGDYAMDYWGQGTSVTVSS

SEQ ID NO: 2 - protein, 107 aa, Artificial sequence
  Murine antibody 3D8.2.3 light chain variable region
DIKMTQSPSSMYASLGERVTITCKASQDINSYLSWFQQKPGKSPKTLIYRANRLVDGVPSRFSGSGSGQDYSLTISSLEYEDMGIYYCLQYDEFPYTFGGGTNLEIK

SEQ ID NO: 3 - protein, 118 aa, Artificial sequence
  Murine antibody 19F6.2.3 heavy chain variable region
DVQLQESGPGLVKPSQSLSLTCTVTGYSITSDYAWNWIRQFPGNKLEWMGYISYSGSIRYNPSLKSRISITRDTSKNQFFLQLNSVTTEDTATYYCARGEITYYFDYWGQGTTLTVSS

SEQ ID NO: 4 - protein, 107 aa, Artificial sequence
  Murine antibody 19F6.2.3 light chain variable region
DIKMTQSPASLSMAIGEKVTIRCITTTDIDDDMNWYQQKPGEPPKLLISEGNTLRPGVPSRFSSSGYGTDFVFTIENMVSEDVADYYCLQSNDLPLTFGAGTKLELK

SEQ ID NO: 5 - protein, 120 aa, Artificial sequence
  Murine antibody 38F8.1.1 heavy chain variable region
EVKLVESGGDLVKPGGSLKLSCTASGFTFSNYAMSWVRQTPEKRLEWVASISSGGPTYYPDSVKGRFTVSRDNARNILYLQMSSLRSEDTAMYYCARGYRYDVNWYFDVWGAGTSVTVSS

SEQ ID NO: 6 - protein, 107 aa, Artificial sequence
  Murine antibody 38F8.1.1 light chain variable region
DIKMTQSPSSMYASLGERVTITCKASQDINSYLTWFQQKPGKSPKTLIHRANRLVDGVPSRFSGSGSGQDYSLTISSLEYEDMGIYYCLQYDEFPYTFGGGTKLEIK

SEQ ID NO: 7 - protein, 8 aa, Artificial sequence
  [IMGT]3D8.2.3/3D8-HuC24/3D8-Hu25/3D8-Hu26/3D8-Hu27/3D8-HuC44/3D8- Hu45/3D8-Hu46/3D8-Hu47/3D8-HuC54/3D8-Hu55/3D8-Hu56/3D8-Hu57/3D8-H uC84/3D8-Hu85/3D8-Hu86/3D8-Hu87/3D8-HuC94/3D8-Hu95/3D8-Hu96/3D8-H u97 CDR-H1
GFTFSSYA

SEQ ID NO: 8 - protein, 7 aa, Artificial sequence
  [IMGT]3D8.2.3/3D8-HuC24/3D8-Hu25/3D8-Hu26/3D8-Hu27/3D8-HuC44/3D8- Hu45/3D8-Hu46/3D8-Hu47/3D8-HuC54/3D8-Hu55/3D8-Hu56/3D8-Hu57 CDR-H2
INSGGST

SEQ ID NO: 9 - protein, 7 aa, Artificial sequence
  [IMGT]3D8-HuC84/3D8-Hu85/3D8-Hu86/3D8-Hu87 CDR-H2
ISSGGST

SEQ ID NO: 10 - protein, 7 aa, Artificial sequence
  [IMGT]3D8-HuC94/3D8-Hu95/3D8-Hu96/3D8-Hu97 CDR-H2
ISNGGST

SEQ ID NO: 11 - protein, 15 aa, Artificial sequence
  [IMGT]3D8.2.3/3D8-HuC24/3D8-Hu25/3D8-Hu26/3D8-Hu27/3D8-HuC44/3D8- Hu45/3D8-Hu46/3D8-Hu47/3D8-HuC54/3D8-Hu55/3D8-Hu56/3D8-Hu57/3D8-H uC84/3D8-Hu85/3D8-Hu86/3D8-Hu87/3D8-HuC94/3D8-Hu95/3D8-Hu96/3D8-H u97 CDR-H3
ARVNYYGYGDYAMDY

SEQ ID NO: 12 - protein, 6 aa, Artificial sequence
  [IMGT]3D8.2.3/3D8-Hu25/3D8-Hu26/3D8-Hu45/3D8-Hu46/3D8-Hu55/3D8-Hu 56/3D8-Hu85/3D8-Hu86/3D8-Hu95/3D8-Hu96 CDR-L1
QDINSY

SEQ ID NO: 13 - protein, 6 aa, Artificial sequence
  [IMGT]3D8-HuC24/3D8-HuC44/3D8-HuC54/3D8-HuC84/3D8-HuC94/3D8-Hu27/ 3D8-Hu47/3D8-Hu57/3D8-Hu87/3D8-Hu97 CDR-L1
QDISNY

SEQ ID NO: 14 - protein, 3 aa, Artificial sequence
  [IMGT]3D8.2.3/3D8-HuC24/3D8-Hu25/3D8-Hu26/3D8-Hu27/3D8-HuC44/3D8- Hu45/3D8-Hu46/3D8-Hu47/3D8-HuC54/3D8-Hu55/3D8-Hu56/3D8-Hu57/3D8-H uC84/3D8-Hu85/3D8-Hu86/3D8-Hu87/3D8-HuC94/3D8-Hu95/3D8-Hu96/3D8-H u97 CDR-L2
RAN

SEQ ID NO: 15 - protein, 9 aa, Artificial sequence
  [IMGT/Abm/Kabat/Chothia]3D8.2.3/3D8-HuC24/ 3D8-Hu25, etc. CDR-L3
LQYDEFPYT

SEQ ID NO: 16 - protein, 10 aa, Artificial sequence
  [AbM]3D8.2.3/3D8-HuC24/3D8-Hu25/3D8-Hu26/3D8-Hu27/3D8-HuC44/3D8-H u45/3D8-Hu46/3D8-Hu47/3D8-HuC54/3D8-Hu55/3D8-Hu56/3D8-Hu57/3D8-Hu C84/3D8-Hu85/3D8-Hu86/3D8-Hu87/3D8-HuC94/3D8-Hu95/3D8-Hu96/3D8-Hu 97 CDR-H1
GFTFSSYAMS

SEQ ID NO: 17 - protein, 9 aa, Artificial sequence
  [AbM]3D8.2.3/3D8-HuC24/3D8-Hu25/3D8-Hu26/3D8-Hu27/3D8-HuC44/3D8-H u45/3D8-Hu46/3D8-Hu47/3D8-HuC54/3D8-Hu55/3D8-Hu56/3D8-Hu57 CDR-H2
SINSGGSTY

SEQ ID NO: 18 - protein, 9 aa, Artificial sequence
  [AbM]3D8-HuC84/3D8-Hu85/3D8-Hu86/3D8-Hu87 CDR-H2
SISSGGSTY

SEQ ID NO: 19 - protein, 9 aa, Artificial sequence
  [AbM]3D8-HuC94/3D8-Hu95/3D8-Hu96/3D8-Hu97 CDR-H2
SISNGGSTY

SEQ ID NO: 20 - protein, 13 aa, Artificial sequence
  [AbM/Kabat/Chothia]3D8.2.3/3D8-HuC24/3D8-Hu25/3D8-Hu26/3D8-Hu27/3 D8-HuC44/3D8-Hu45/3D8-Hu46/3D8-Hu47/3D8-HuC54/3D8-Hu55/3D8-Hu56/3 D8-Hu57/3D8-HuC84/3D8-Hu85/3D8-Hu86/3D8-Hu87/3D8-HuC94/3D8-Hu95/3 D8-Hu96/3D8-Hu97 CDR-H3
VNYYGYGDYAMDY

SEQ ID NO: 21 - protein, 11 aa, Artificial sequence
  [AbM/Kabat/Chothia]3D8.2.3 CDR-L1
KASQDINSYLS

SEQ ID NO: 22 - protein, 11 aa, Artificial sequence
  [AbM/Kabat/Chothia]3D8-Hu25/3D8-Hu26/3D8-Hu45/3D8-Hu46/3D8-Hu55/3 D8-Hu56/3D8-Hu85/3D8-Hu86/3D8-Hu95/3D8-Hu96 CDR-L1
QASQDINSYLS

SEQ ID NO: 23 - protein, 11 aa, Artificial sequence
  [AbM/Kabat/Chothia]3D8-Hu27/3D8-Hu47/3D8-Hu57/3D8-Hu87/3D8-Hu97 CDR-L1
QASQDISNYLS

SEQ ID NO: 24 - protein, 7 aa, Artificial sequence
  [AbM/Kabat/Chothia]3D8.2.3/38F8.1.1 CDR-L2
RANRLVD

SEQ ID NO: 25 - protein, 7 aa, Artificial sequence
  [AbM/Kabat/Chothia]3D8-HuC24/3D8-HuC44/3D8-HuC54/3D8-HuC84/3D8-Hu C94/3D8-Hu25/3D8-Hu26/3D8-Hu27/3D8-Hu45/3D8-Hu46/3D8-Hu47/3D8-Hu5 5/3D8-Hu56/3D8-Hu57/3D8-Hu85/3D8-Hu86/3D8-Hu87/3D8-Hu95/3D8-Hu96/ 3D8-Hu97 CDR-L2
RANRLVT

SEQ ID NO: 26 - DNA, 321 bp, Artificial sequence
  Nucleotide sequence of human kappa light chain constant region
cgtacggtggctgcaccatctgtcttcatcttcccgccatctgatgagcagttgaaatctggaactgcctctgttgtgtgcctgctgaataacttctatccccgcgaggccaaagtacagtggaaggtggataacgccctccaatcgggtaactcccaggagagtgtcacagagcaggacagcaaggacagcacctacagcctcagcagcaccctgacgctgagcaaagcagactacgagaaacacaaagtctacgcctgcgaagtcacccatcagggcctgagctcgcccgtcacaaagagcttcaaccgcggagagtgt

SEQ ID NO: 27 - protein, 5 aa, Artificial sequence
  [Kabat]3D8.2.3/3D8-HuC24/3D8-Hu25/3D8-Hu26/3D8-Hu27/3D8-HuC44/3D8 -Hu45/3D8-Hu46/3D8-Hu47/3D8-HuC54/3D8-Hu55/3D8-Hu56/3D8-Hu57/3D8- HuC84/3D8-Hu85/3D8-Hu86/3D8-Hu87/3D8-HuC94/3D8-Hu95/3D8-Hu96/3D8- Hu97 CDR-H1
SYAMS

SEQ ID NO: 28 - protein, 16 aa, Artificial sequence
  [Kabat]3D8.2.3/3D8-HuC24/3D8-Hu25/3D8-Hu26/3D8-Hu27/3D8-HuC44/3D8 -Hu45/3D8-Hu46/3D8-Hu47/3D8-HuC54/3D8-Hu55/3D8-Hu56/3D8-Hu57 CDR-H2
SINSGGSTYYPDSVKG

SEQ ID NO: 29 - protein, 16 aa, Artificial sequence
  [Kabat]3D8-HuC84/3D8-Hu85/3D8-Hu86/3D8-Hu87 CDR-H2
SISSGGSTYYPDSVKG

SEQ ID NO: 30 - protein, 16 aa, Artificial sequence
  [Kabat]3D8-HuC94/3D8-Hu95/3D8-Hu96/3D8-Hu97 CDR-H2
SISNGGSTYYPDSVKG

SEQ ID NO: 31 - protein, 7 aa, Artificial sequence
  [Chothia]3D8.2.3/3D8-HuC24/3D8-Hu25/3D8-Hu26/3D8-Hu27/3D8-HuC44/3 D8-Hu45/3D8-Hu46/3D8-Hu47/3D8-HuC54/3D8-Hu55/3D8-Hu56/3D8-Hu57/3D 8-HuC84/3D8-Hu85/3D8-Hu86/3D8-Hu87/3D8-HuC94/3D8-Hu95/3D8-Hu96/3D 8-Hu97 CDR-H1
GFTFSSY

SEQ ID NO: 32 - protein, 5 aa, Artificial sequence
  [Chothia]3D8.2.3/3D8-HuC24/3D8-Hu25/3D8-Hu26/3D8-Hu27/3D8-HuC44/3 D8-Hu45/3D8-Hu46/3D8-Hu47/3D8-HuC54/3D8-Hu55/3D8-Hu56/3D8-Hu57 CDR-H2
NSGGS

SEQ ID NO: 33 - protein, 5 aa, Artificial sequence
  [Chothia]3D8-HuC84/3D8-Hu85/3D8-Hu86/3D8-Hu87 CDR-H2
SSGGS

SEQ ID NO: 34 - protein, 5 aa, Artificial sequence
  [Chothia]3D8-HuC94/3D8-Hu95/3D8-Hu96/3D8-Hu97 CDR-H2
SNGGS

SEQ ID NO: 35 - protein, 9 aa, Artificial sequence
  [IMGT]19F6.2.3/19F6-Hu11/19F6-Hu12, etc. CDR-H1
GYSITSDYA

SEQ ID NO: 36 - protein, 7 aa, Artificial sequence
  [IMGT]19F6.2.3/19F6-Hu11/19F6-Hu12, etc. CDR-H2
ISYSGSI

SEQ ID NO: 37 - protein, 11 aa, Artificial sequence
  [IMGT]19F6.2.3/19F6-Hu11/19F6-Hu12, etc. CDR-H3
ARGEITYYFDY

SEQ ID NO: 38 - protein, 6 aa, Artificial sequence
  [IMGT]19F6.2.3/19F6-Hu11/19F6-Hu12/19F6-Hu13/19F6-Hu14/19F6-Hu15/ 19F6-Hu21/19F6-Hu22/19F6-Hu23/19F6-Hu24/19F6-Hu25/19F6-Hu31/19F6- Hu32/19F6-Hu33/19F6-Hu34/19F6-Hu35/19F6-Hu35V5 CDR-L1
TDIDDD

SEQ ID NO: 39 - protein, 6 aa, Artificial sequence
  [IMGT]19F6-Hu35V1/19F6-Hu35V3/19F6-Hu35V7/19F6-Hu35V9 CDR-L1
TSIDDD

SEQ ID NO: 40 - protein, 6 aa, Artificial sequence
  [IMGT]19F6-Hu35V2/19F6-Hu35V10 CDR-L1
TDIDSD

SEQ ID NO: 41 - protein, 6 aa, Artificial sequence
  [IMGT]19F6-Hu35V4 CDR-L1
TSIDND

SEQ ID NO: 42 - protein, 6 aa, Artificial sequence
  [IMGT]19F6-Hu35V6/19F6-Hu35V8 CDR-L1
TDIDND

SEQ ID NO: 43 - protein, 3 aa, Artificial sequence
  [IMGT]19F6.2.3/19F6-Hu11/19F6-Hu12, etc. CDR-L2
EGN

SEQ ID NO: 44 - protein, 9 aa, Artificial sequence
  [IMGT/Abm/Kabat/Chothia]19F6.2.3/19F6-Hu11/19F6-Hu12, etc. CDR-L3
LQSNDLPLT

SEQ ID NO: 45 - protein, 11 aa, Artificial sequence
  [AbM]19F6.2.3/19F6-Hu11/19F6-Hu12, etc. CDR-H1
GYSITSDYAWN

SEQ ID NO: 46 - protein, 9 aa, Artificial sequence
  [AbM]19F6.2.3/19F6-Hu11/19F6-Hu12, etc. CDR-H2
YISYSGSIR

SEQ ID NO: 47 - protein, 9 aa, Artificial sequence
  [AbM/Kabat/Chothia]19F6.2.3/19F6-Hu11/19F6-Hu12, etc. CDR-H3
GEITYYFDY

SEQ ID NO: 48 - protein, 11 aa, Artificial sequence
  [AbM/Kabat/Chothia]19F6.2.3/19F6-Hu11/19F6-Hu12/19F6-Hu21/19F6-Hu 22/19F6-Hu31/19F6-Hu32 CDR-L1
ITTTDIDDDMN

SEQ ID NO: 49 - protein, 11 aa, Artificial sequence
  [AbM/Kabat/Chothia]19F6-Hu13/19F6-Hu23/19F6-Hu33 CDR-L1
RASTDIDDDMN

SEQ ID NO: 50 - protein, 11 aa, Artificial sequence
  [AbM/Kabat/Chothia]19F6-Hu14/19F6-Hu24/19F6-Hu34 CDR-L1
QTSTDIDDDLN

SEQ ID NO: 51 - protein, 11 aa, Artificial sequence
  [AbM/Kabat/Chothia]19F6-Hu15/19F6-Hu25/19F6-Hu35/19F6-Hu35V5 CDR-L1
KASTDIDDDMN

SEQ ID NO: 52 - protein, 11 aa, Artificial sequence
  [AbM/Kabat/Chothia]19F6-Hu35V1/19F6-Hu35V3/19F6-Hu35V7/19F6-Hu35V 9 CDR-L1
KASTSIDDDMN

SEQ ID NO: 53 - protein, 11 aa, Artificial sequence
  [AbM/Kabat/Chothia]19F6-Hu35V2/19F6-Hu35V10 CDR-L1
KASTDIDSDMN

SEQ ID NO: 54 - protein, 11 aa, Artificial sequence
  [AbM/Kabat/Chothia]19F6-Hu35V4 CDR-L1
KASTSIDNDMN

SEQ ID NO: 55 - protein, 11 aa, Artificial sequence
  [AbM/Kabat/Chothia]19F6-Hu35V6/19F6-Hu35V8 CDR-L1
KASTDIDNDMN

SEQ ID NO: 56 - protein, 7 aa, Artificial sequence
  [AbM/Kabat/Chothia]19F6.2.3/19F6-Hu11/19F6-Hu15/19F6-Hu21/19F6-Hu 25/19F6-Hu31/19F6-Hu35/19F6-Hu35V1/19F6-Hu35V2/19F6-Hu35V3/19F6-H u35V4/19F6-Hu35V5/19F6-Hu35V6/19F6-Hu35V7/19F6-Hu35V8/19F6-Hu35V9 /19F6-Hu35V10 CDR-L2
EGNTLRP

SEQ ID NO: 57 - protein, 7 aa, Artificial sequence
  [AbM/Kabat/Chothia]19F6-Hu12/19F6-Hu13/19F6-Hu22/19F6-Hu23/19F6-H u32/19F6-Hu33 CDR-L2
EGNTLQS

SEQ ID NO: 58 - protein, 7 aa, Artificial sequence
  [AbM/Kabat/Chothia]19F6-Hu14/19F6-Hu24/19F6-Hu34 CDR-L2
EGNTLET

SEQ ID NO: 59 - DNA, 990 bp, Artificial sequence
  Human IgG1 heavy chain constant region nucleotide sequence
gctagcaccaagggacccagcgttttccctctggctccatcctccaagagcacctctggtggaacagctgctctgggctgcctggtcaaggactactttcctgagcctgtgaccgtgtcctggaactctggcgctctgacatctggcgtgcacacctttccagctgtgctgcagtcctctggcctgtactctctgtcctccgtcgtgaccgtgccttctagctctctgggcacccagacctacatctgcaatgtgaaccacaagccttccaacaccaaggtggacaagaaggtggaacccaagtcctgcgacaagacccacacctgtcctccatgtcctgctccagaactgctcggcggaccttccgtgttcctgtttcctccaaagcctaaggacaccctgatgatctctcggacccctgaagtgacctgcgtggtggtggatgtgtctcacgaggacccagaagtgaagttcaattggtacgtggacggcgtggaagtgcacaacgccaagaccaagcctagagaggaacagtacaactccacctacagagtggtgtccgtgctgaccgtgctgcaccaggattggctgaacggcaaagagtacaagtgcaaggtgtccaacaaggccctgcctgctcctatcgaaaagaccatctccaaggccaagggccagcctagggaaccccaggtttacaccttgcctccatctcgggacgagctgaccaagaaccaggtgtccctgacctgtctcgtgaagggcttctacccctccgatatcgccgtggaatgggagtctaatggccagcctgagaacaactacaagacaacccctcctgtgctggactccgacggctcattcttcctgtactccaagctgacagtggacaagtccagatggcagcagggcaacgtgttctcctgctccgtgatgcacgaggccctgcacaatcactacacacagaagtccctgtctctgtcccctggcaag

SEQ ID NO: 60 - protein, 6 aa, Artificial sequence
  [Kabat]19F6.2.3/19F6-Hu11/19F6-Hu12, etc. CDR-H1
SDYAWN

SEQ ID NO: 61 - protein, 16 aa, Artificial sequence
  [Kabat]19F6.2.3/19F6-Hu31/19F6-Hu32/19F6-Hu33/19F6-Hu34/19F6-Hu35 /19F6-Hu35V1/19F6-Hu35V2/19F6-Hu35V3/19F6-Hu35V4/19F6-Hu35V5/19F6 -Hu35V6/19F6-Hu35V7/19F6-Hu35V8/19F6-Hu35V9/19F6-Hu35V10 CDR-H2
YISYSGSIRYNPSLKS

SEQ ID NO: 62 - protein, 16 aa, Artificial sequence
  [Kabat]19F6-Hu11/19F6-Hu12/19F6-Hu13/19F6-Hu14/19F6-Hu15 CDR-H2
YISYSGSIRYKPSLKD

SEQ ID NO: 63 - protein, 16 aa, Artificial sequence
  [Kabat]19F6-Hu21/19F6-Hu22/19F6-Hu23/19F6-Hu24/19F6-Hu25 CDR-H2
YISYSGSIRYNPSLKD

SEQ ID NO: 64 - protein, 8 aa, Artificial sequence
  [Chothia]19F6.2.3/19F6-Hu11/19F6-Hu12, etc. CDR-H1
GYSITSDY

SEQ ID NO: 65 - protein, 5 aa, Artificial sequence
  [Chothia]19F6.2.3/19F6-Hu11/19F6-Hu12, etc. CDR-H2
SYSGS

SEQ ID NO: 66 - protein, 8 aa, Artificial sequence
  [IMGT]38F8.1.1/38F8-Hu14/38F8-Hu16/38F8-Hu17/38F8-Hu18/38F8-Hu24/ 38F8-Hu26/38F8-Hu27/38F8-Hu28/38F8-Hu34/38F8-Hu36/38F8-Hu37/38F8- Hu38/38F8-Hu54/38F8-Hu56/38F8-Hu57/38F8-Hu58/38F8-Hu64/38F8-Hu66/ 38F8-Hu67/38F8-Hu68 CDR-H1
GFTFSNYA

SEQ ID NO: 67 - protein, 7 aa, Artificial sequence
  [IMGT]38F8.1.1/38F8-Hu14/38F8-Hu16/38F8-Hu17/38F8-Hu18/38F8-Hu24/ 38F8-Hu26/38F8-Hu27/38F8-Hu28/38F8-Hu34/38F8-Hu36/38F8-Hu37/38F8- Hu38/38F8-Hu54/38F8-Hu56/38F8-Hu57/38F8-Hu58/38F8-Hu64/38F8-Hu66/ 38F8-Hu67/38F8-Hu68 CDR-H2
ISSGGPT

SEQ ID NO: 68 - protein, 14 aa, Artificial sequence
  [IMGT]38F8.1.1/38F8-Hu14/38F8-Hu16/38F8-Hu17/38F8-Hu18/38F8-Hu24/ 38F8-Hu26/38F8-Hu27/38F8-Hu28/38F8-Hu34/38F8-Hu36/38F8-Hu37/38F8- Hu38/38F8-Hu54/38F8-Hu56/38F8-Hu57/38F8-Hu58/38F8-Hu64/38F8-Hu66/ 38F8-Hu67/38F8-Hu68 CDR-H3
ARGYRYDVNWYFDV

SEQ ID NO: 69 - protein, 6 aa, Artificial sequence
  [IMGT]38F8.1.1/38F8-Hu16/38F8-Hu18/38F8-Hu26/38F8-Hu28/38F8-Hu36/ 38F8-Hu38/38F8-Hu56/38F8-Hu58/38F8-Hu66/38F8-Hu68 CDR-L1
QDINSY

SEQ ID NO: 70 - protein, 6 aa, Artificial sequence
  [IMGT]38F8-Hu14/38F8-Hu24/38F8-Hu34/38F8-Hu54/38F8-Hu64/38F8-Hu17 /38F8-Hu27/38F8-Hu37/38F8-Hu57/38F8-Hu67 CDR-L1
QDISNY

SEQ ID NO: 71 - protein, 3 aa, Artificial sequence
  [IMGT]38F8.1.1/38F8-Hu14/38F8-Hu16/38F8-Hu17/38F8-Hu18/38F8-Hu24/ 38F8-Hu26/38F8-Hu27/38F8-Hu28/38F8-Hu34/38F8-Hu36/38F8-Hu37/38F8- Hu38/38F8-Hu54/38F8-Hu56/38F8-Hu57/38F8-Hu58/38F8-Hu64/38F8-Hu66/ 38F8-Hu67/38F8-Hu68 CDR-L2
RAN

SEQ ID NO: 72 - protein, 10 aa, Artificial sequence
  [AbM]38F8.1.1/38F8-Hu14/38F8-Hu16/38F8-Hu17/38F8-Hu18/38F8-Hu24/3 8F8-Hu26/38F8-Hu27/38F8-Hu28/38F8-Hu34/38F8-Hu36/38F8-Hu37/38F8-H u38/38F8-Hu54/38F8-Hu56/38F8-Hu57/38F8-Hu58/38F8-Hu64/38F8-Hu66/3 8F8-Hu67/38F8-Hu68 CDR-H1
GFTFSNYAMS

SEQ ID NO: 73 - protein, 9 aa, Artificial sequence
  [AbM]38F8.1.1/38F8-Hu14/38F8-Hu16/38F8-Hu17/38F8-Hu18/38F8-Hu24/3 8F8-Hu26/38F8-Hu27/38F8-Hu28/38F8-Hu34/38F8-Hu36/38F8-Hu37/38F8-H u38/38F8-Hu54/38F8-Hu56/38F8-Hu57/38F8-Hu58/38F8-Hu64/38F8-Hu66/3 8F8-Hu67/38F8-Hu68 CDR-H2
SISSGGPTY

SEQ ID NO: 74 - protein, 12 aa, Artificial sequence
  [AbM/Kabat/Chothia]38F8.1.1/38F8-Hu14/38F8-Hu16/38F8-Hu17/38F8-Hu 18/38F8-Hu24/38F8-Hu26/38F8-Hu27/38F8-Hu28/38F8-Hu34/38F8-Hu36/38 F8-Hu37/38F8-Hu38/38F8-Hu54/38F8-Hu56/38F8-Hu57/38F8-Hu58/38F8-Hu 64/38F8-Hu66/38F8-Hu67/38F8-Hu68 CDR-H3
GYRYDVNWYFDV

SEQ ID NO: 75 - protein, 11 aa, Artificial sequence
  [AbM/Kabat/Chothia]38F8.1.1 CDR-L1
KASQDINSYLT

SEQ ID NO: 76 - protein, 11 aa, Artificial sequence
  [AbM/Kabat/Chothia]38F8-Hu16/38F8-Hu18/38F8-Hu26/38F8-Hu28/38F8-H u36/38F8-Hu38/38F8-Hu56/38F8-Hu58/38F8-Hu66/38F8-Hu68 CDR-L1
QASQDINSYLT

SEQ ID NO: 77 - protein, 11 aa, Artificial sequence
  [AbM/Kabat/Chothia]3D8-HuC24/3D8-HuC44/3D8-HuC54/3D8-HuC84/3D8-Hu C94/38F8-Hu14/38F8-Hu24/38F8-Hu34/38F8-Hu54/38F8-Hu64/38F8-Hu17/3 8F8-Hu27/38F8-Hu37/38F8-Hu57/38F8-Hu67 CDR-L1
QASQDISNYLT

SEQ ID NO: 78 - protein, 7 aa, Artificial sequence
  [AbM/Kabat/Chothia]38F8-Hu14/38F8-Hu24/38F8-Hu34/38F8-Hu54/38F8-H u64/38F8-Hu16/38F8-Hu17/38F8-Hu18/38F8-Hu26/38F8-Hu27/38F8-Hu28/3 8F8-Hu36/38F8-Hu37/38F8-Hu38/38F8-Hu56/38F8-Hu57/38F8-Hu58/38F8-H u66/38F8-Hu67/38F8-Hu68 CDR-L2
RANRLVT

SEQ ID NO: 79 - protein, 5 aa, Artificial sequence
  [Kabat]38F8.1.1/38F8-Hu14/38F8-Hu16/38F8-Hu17/38F8-Hu18/38F8-Hu24 /38F8-Hu26/38F8-Hu27/38F8-Hu28/38F8-Hu34/38F8-Hu36/38F8-Hu37/38F8 -Hu38/38F8-Hu54/38F8-Hu56/38F8-Hu57/38F8-Hu58/38F8-Hu64/38F8-Hu66 /38F8-Hu67/38F8-Hu68 CDR-H1
NYAMS

SEQ ID NO: 80 - protein, 16 aa, Artificial sequence
  [Kabat]38F8.1.1/38F8-Hu24/38F8-Hu26/38F8-Hu27/38F8-Hu28/38F8-Hu54 /38F8-Hu56/38F8-Hu57/38F8-Hu58/38F8-Hu64/38F8-Hu66/38F8-Hu67/38F8 -Hu68 CDR-H2
SISSGGPTYYPDSVKG

SEQ ID NO: 81 - protein, 16 aa, Artificial sequence
  [Kabat]38F8-Hu14/38F8-Hu16/38F8-Hu17/38F8-Hu18/38F8-Hu34/38F8-Hu3 6/38F8-Hu37/38F8-Hu38 CDR-H2
SISSGGPTYYADSVKG

SEQ ID NO: 82 - protein, 7 aa, Artificial sequence
  [Chothia]38F8.1.1/38F8-Hu14/38F8-Hu16/38F8-Hu17/38F8-Hu18/38F8-Hu 24/38F8-Hu26/38F8-Hu27/38F8-Hu28/38F8-Hu34/38F8-Hu36/38F8-Hu37/38 F8-Hu38/38F8-Hu54/38F8-Hu56/38F8-Hu57/38F8-Hu58/38F8-Hu64/38F8-Hu 66/38F8-Hu67/38F8-Hu68 CDR-H1
GFTFSNY

SEQ ID NO: 83 - protein, 5 aa, Artificial sequence
  [Chothia]38F8.1.1/38F8-Hu14/38F8-Hu16/38F8-Hu17/38F8-Hu18/38F8-Hu 24/38F8-Hu26/38F8-Hu27/38F8-Hu28/38F8-Hu34/38F8-Hu36/38F8-Hu37/38 F8-Hu38/38F8-Hu54/38F8-Hu56/38F8-Hu57/38F8-Hu58/38F8-Hu64/38F8-Hu 66/38F8-Hu67/38F8-Hu68 CDR-H2
SSGGP

SEQ ID NO: 84 - protein, 118 aa, Artificial sequence
  Humanized antibody 19F6-Hu11/19F6-Hu12/19F6-Hu13/19F6-Hu14/19F6-Hu15 heavy chain variable region
QVQLQESGPGLVKPSETLSLTCTVTGYSITSDYAWNWIRQPPGKGLEWMGYISYSGSIRYKPSLKDRITISRDTSKNQFSLKLSSVTAADTAVYYCARGEITYYFDYWGQGTLVTVSS

SEQ ID NO: 85 - protein, 118 aa, Artificial sequence
  Humanized antibody 19F6-Hu21/19F6-Hu22/19F6-Hu23/19F6-Hu24/19F6-Hu25 heavy chain
QVQLQESGPGLVKPSETLSLTCTVSGYSITSDYAWNWIRQPPGKGLEWMGYISYSGSIRYNPSLKDRITISRDTSKNQFSLKLSSVTAADTAVYYCARGEITYYFDYWGQGTLVTVSS

SEQ ID NO: 86 - protein, 118 aa, Artificial sequence
  Humanized antibody 19F6-Hu31/19F6-Hu32/19F6-Hu33/19F6-Hu34/19F6-Hu35/19F6-Hu35V1/19F 6-Hu35V2/19F6-Hu35V3/19F6-Hu35V4/19F6-Hu35V5/19F6-Hu35V6/19F6-Hu3 5V7/19F6-Hu35V8/19F6-Hu35V9/19F6-Hu35V10 VH
QVQLQESGPGLVKPSQTLSLTCTVSGYSITSDYAWNWIRQFPGKGLEWIGYISYSGSIRYNPSLKSRVTISRDTSKNQFSLKLSSVTAADTAVYYCARGEITYYFDYWGQGTLVTVSS

SEQ ID NO: 87 - protein, 107 aa, Artificial sequence
  Humanized antibody 19F6-Hu11/19F6-Hu21/19F6-Hu31 light chain variable region
DIQMTQSPSSLSASVGDRVTITCITTTDIDDDMNWYQQKPGKAPKLLISEGNTLRPGVPSRFSGSGYGTDFTLTISSLQPEDFATYYCLQSNDLPLTFGQGTKLEIK

SEQ ID NO: 88 - protein, 107 aa, Artificial sequence
  Humanized antibody 19F6-Hu12/19F6-Hu22/19F6-Hu32 light chain variable region
DIQMTQSPSSLSASVGDRVTITCITTTDIDDDMNWYQQKPGKAPKLLISEGNTLQSGVPSRFSGSGYGTDFTLTISSLQPEDFATYYCLQSNDLPLTFGQGTKLEIK

SEQ ID NO: 89 - protein, 107 aa, Artificial sequence
  Humanized antibody 19F6-Hu13/19F6-Hu23/19F6-Hu33 light chain variable region
DIQMTQSPSSLSASVGDRVTITCRASTDIDDDMNWYQQKPGKAPKLLIYEGNTLQSGVPSRFSGSGYGTDFTLTISSLQPEDFATYYCLQSNDLPLTFGQGTKLEIK

SEQ ID NO: 90 - protein, 107 aa, Artificial sequence
  Humanized antibody 19F6-Hu14/19F6-Hu24/19F6-Hu34 light chain variable region
DIQMTQSPSSLSASVGDRVTITCQTSTDIDDDLNWYQQKPGKPPKLLISEGNTLETGVPSRFSGSGSGTDFTFTISSLQPEDIADYYCLQSNDLPLTFGAGTKLEIK

SEQ ID NO: 91 - protein, 107 aa, Artificial sequence
  Humanized antibody 19F6-Hu15/19F6-Hu25/19F6-Hu35 light chain variable region
ETTLTQSPAFMSATPGDKVTISCKASTDIDDDMNWYQQKPGEPPKLIISEGNTLRPGIPPRFSSSGYGTDFTFTINNIESEDAADYYCLQSNDLPLTFGQGTKLEIK

SEQ ID NO: 92 - protein, 107 aa, Artificial sequence
  Humanized antibody 19F6-Hu35V1 light chain variable region
ETTLTQSPAFMSATPGDKVTISCKASTSIDDDMNWYQQKPGEPPKLIISEGNTLRPGIPPRFSSSGYGTDFTFTINKIKSEDAATYYCLQSNDLPLTFGQGTKLEIK

SEQ ID NO: 93 - protein, 107 aa, Artificial sequence
  Humanized antibody 19F6-Hu35V2 light chain variable region
ETTLTQSPAFMSATPGDKVTISCKASTDIDSDMNWYQQKPGEPPKLIISEGNTLRPGIPPRFSSSGYGTDFTFTINKIKSEDAATYYCLQSNDLPLTFGQGTKLEIK

SEQ ID NO: 94 - protein, 107 aa, Artificial sequence
  Humanized antibody 19F6-Hu35V3 light chain variable region
ETTLTQSPAFMSATPGDKVTISCKASTSIDDDMNWYQQKPGKPPKLIISEGNTLRPGIPPRFSSSGYGTDFTFTINKIESEDAATYYCLQSNDLPLTFGQGTKLEIK

SEQ ID NO: 95 - protein, 107 aa, Artificial sequence
  Humanized antibody 19F6-Hu35V4 light chain variable region
ETTLTQSPAFMSATPGDKVTISCKASTSIDNDMNWYQQKPGKPPKLIISEGNTLRPGIPPRFSSSGYGTDFTFTINKIESEDAATYYCLQSNDLPLTFGQGTKLEIK

SEQ ID NO: 96 - protein, 107 aa, Artificial sequence
  Humanized antibody 19F6-Hu35V5 light chain variable region
ETTLTQSPAFMSATPGDKVTISCKASTDIDDDMNWYQQKPGKPPKLIISEGNTLRPGIPPRFSSSGYGTDFTFTINNIKSEDAATYYCLQSNDLPLTFGQGTKLEIK

SEQ ID NO: 97 - protein, 107 aa, Artificial sequence
  Humanized antibody 19F6-Hu35V6 light chain variable region
ETTLTQSPAFMSATPGDKVTISCKASTDIDNDMNWYQQKPGKPPKLIISEGNTLRPGIPPRFSSSGYGTDFTFTINNIKSEDAATYYCLQSNDLPLTFGQGTKLEIK

SEQ ID NO: 98 - protein, 107 aa, Artificial sequence
  Humanized antibody 19F6-Hu35V7 light chain variable region
ETTLTQSPAFMSATPGDKVTISCKASTSIDDDMNWYQQKPGKPPKLIISEGNTLRPGIPPRFSSSGYGTDFTFTINNIQSEDAATYYCLQSNDLPLTFGQGTKLEIK

SEQ ID NO: 99 - protein, 107 aa, Artificial sequence
  Humanized antibody 19F6-Hu35V8 light chain variable region
ETTLTQSPAFMSATPGDKVTISCKASTDIDNDMNWYQQKPGKPPKLIISEGNTLRPGIPPRFSSSGYGTDFTFTINNIQSEDAATYYCLQSNDLPLTFGQGTKLEIK

SEQ ID NO: 100 - protein, 107 aa, Artificial sequence
  Humanized antibody 19F6-Hu35V9 light chain variable region
ETTLTQSPAFMSATPGDKVTISCKASTSIDDDMNWYQQKPGKPPKLIISEGNTLRPGIPPRFSSSGYGTDFTFTIRKIESEDAADYYCLQSNDLPLTFGQGTKLEIK

SEQ ID NO: 101 - protein, 107 aa, Artificial sequence
  Humanized antibody 19F6-Hu35V10 light chain variable region
ETTLTQSPAFMSATPGDKVTISCKASTDIDSDMNWYQQKPGKPPKLIISEGNTLRPGIPPRFSSSGYGTDFTFTIRKIESEDAADYYCLQSNDLPLTFGQGTKLEIK

SEQ ID NO: 102 - protein, 121 aa, Artificial sequence
  Humanized antibody 3D8-HuC24/3D8-Hu25/3D8-Hu26 /3D8-Hu27 heavy chain variable region
EVQLVESGGGLVQPGGSLRLSCAASGFTFSSYAMSWVRQAPGKGLEWVASINSGGSTYYPDSVKGRFTISRDNAKNSLYLQMNSLRAEDTAVYYCARVNYYGYGDYAMDYWGQGTLVTVSS

SEQ ID NO: 103 - protein, 121 aa, Artificial sequence
  Humanized antibody 3D8-HuC44/3D8-Hu45/3D8-Hu46 /3D8-Hu47 heavy chain variable region
EVQLVESGGGLVQPGGSLRLSCAASGFTFSSYAMSWVRQAPGKGLEWVSSINSGGSTYYPDSVKGRFTISRDNSKNTLYLQMNSLRAEDTAVYYCARVNYYGYGDYAMDYWGQGTLVTVSS

SEQ ID NO: 104 - protein, 121 aa, Artificial sequence
  Humanized antibody 3D8-HuC 54/3D8-Hu55/3D8-Hu56 /3D8-Hu57 heavy chain variable region
EVQLVESGGGLVQPGGSLRLSCAASGFTFSSYAMSWVRQAPGKGLEWVSSINSGGSTYYPDSVKGRFTISRENAKNSLYLQMNSLRAGDTAVYYCARVNYYGYGDYAMDYWGQGTLVTVSS

SEQ ID NO: 105 - protein, 121 aa, Artificial sequence
  Humanized antibody 3D8-HuC84/3D8-Hu85/3D8-Hu86 /3D8-Hu87 heavy chain variable region
EVQLVESGGGLVQPGGSLRLSCAASGFTFSSYAMSWVRQAPEKRLEWVSSISSGGSTYYPDSVKGRFTISRDNSKNTLYLQMNSLRAEDTAVYYCARVNYYGYGDYAMDYWGQGTLVTVSS

SEQ ID NO: 106 - protein, 121 aa, Artificial sequence
  Humanized antibody 3D8-HuC94/3D8-Hu95/3D8-Hu96 /3D8-Hu97 heavy chain variable region
EVQLVESGGGLVQPGGSLRLSCAASGFTFSSYAMSWVRQAPEKRLEWVSSISNGGSTYYPDSVKGRFTISRDNSKNTLYLQMNSLRAEDTAVYYCARVNYYGYGDYAMDYWGQGTLVTVSS

SEQ ID NO: 107 - protein, 107 aa, Artificial sequence
  Humanized antibody 3D8-HuC24/3D8-HuC44/3D8-HuC54 /3D8-HuC84/3D8-HuC94/38F8-Hu14/38F8-Hu24/38F8-Hu34/38F8-Hu54/38F8 -Hu64 light chain variable region
DIQMTQSPSSLSASVGDRVTITCQASQDISNYLTWFQQKPGKSPKTLIHRANRLVTGVPSRFSGSGSGTDFTFTISSLQPEDIATYYCLQYDEFPYTFGGGTKVEIK

SEQ ID NO: 108 - protein, 107 aa, Artificial sequence
  Humanized antibody 3D8-Hu25/3D8-Hu45/3D8-Hu55/3D8-Hu85/3D8-Hu95 light chain variable region
DIQMTQSPSSLSASVGDRVTITCQASQDINSYLSWFQQKPGKAPKTLIYRANRLVTGVPSRFSGSGSGTDFTFTISSLQPEDIATYYCLQYDEFPYTFGGGTKLEIK

SEQ ID NO: 109 - protein, 107 aa, Artificial sequence
  Humanized antibody 3D8-Hu26/3D8-Hu46/3D8-Hu56/3D8-Hu86/3D8-Hu96 light chain variable region
DIQMTQSPSSLSASVGDRVTITCQASQDINSYLSWFQQKPGKSPKTLIYRANRLVTGVPSRFSGSGSGTDYTFTISSLQPEDIATYYCLQYDEFPYTFGGGTKLEIK

SEQ ID NO: 110 - protein, 107 aa, Artificial sequence
  Humanized antibody 3D8-Hu27/3D8-Hu47/3D8-Hu57/3D8-Hu87/3D8-Hu97 light chain variable region
DIQMTQSPSSLSASVGDRVTITCQASQDISNYLSWFQQKPGKSPKTLIYRANRLVTGVPSRFSGSGSGTDYTFTISSLQPEDIATYYCLQYDEFPYTFGGGTKLEIK

SEQ ID NO: 111 - protein, 120 aa, Artificial sequence
  Humanized antibody 38F8-Hu14/38F8-Hu16/38F8-Hu17 /38F8-Hu18 heavy chain variable region
EVQLVESGGGLVQPGGSLRLSCTASGFTFSNYAMSWVRQAPGKGLEWVASISSGGPTYYADSVKGRFTVSRDNSRNTLYLQMNSLRAEDTAVYYCARGYRYDVNWYFDVWGRGTLVTVSS

SEQ ID NO: 112 - protein, 120 aa, Artificial sequence
  Humanized antibody 38F8-Hu24/38F8-Hu26/38F8-Hu27 /38F8-Hu28 heavy chain variable region
EVQLVESGGGLVQPGGSLRLSCAASGFTFSNYAMSWVRQAPGKGLEWVASISSGGPTYYPDSVKGRFTVSRDNSKNTLYLQMNSLRAEDTAVYYCARGYRYDVNWYFDVWGAGTMVTVSS

SEQ ID NO: 113 - protein, 120 aa, Artificial sequence
  Humanized antibody 38F8-Hu34/38F8-Hu36/38F8-Hu37 /38F8-Hu38 heavy chain variable region
QVQLVESGGGLVKPGGSLRLSCAASGFTFSNYAMSWVRQAPGKGLEWVASISSGGPTYYADSVKGRFTISRDNAKNSLYLQMNSLRAEDTAVYYCARGYRYDVNWYFDVWGAGTMVTVSS

SEQ ID NO: 114 - protein, 120 aa, Artificial sequence
  Humanized antibody 38F8-Hu54/38F8-Hu56/38F8-Hu57 /38F8-Hu58 heavy chain variable region
EVQLVESGGGLVQPGGSLRLSCAASGFTFSNYAMSWVRQAPEKRLEWVASISSGGPTYYPDSVKGRFTVSRDNSKNTLYLQMNSLRAEDTAVYYCARGYRYDVNWYFDVWGAGTMVTVSS

SEQ ID NO: 115 - protein, 120 aa, Artificial sequence
  Humanized antibody 38F8-Hu64/38F8-Hu66/38F8-Hu67 /38F8-Hu68 heavy chain variable region
QVQLVESGGGLVKPGGSLRLSCAASGFTFSNYAMSWVRQAPEKRLEWVASISSGGPTYYPDSVKGRFTISRDNAKNSLYLQMNSLRAEDTAVYYCARGYRYDVNWYFDVWGAGTMVTVSS

SEQ ID NO: 116 - protein, 107 aa, Artificial sequence
  Humanized antibody 38F8-Hu16/38F8-Hu26/38F8-Hu36 /38F8-Hu56/38F8-Hu66 light chain variable region
DIQMTQSPSSLSASVGDRVTITCQASQDINSYLTWFQQKPGKSPKTLIHRANRLVTGVPSRFSGSGSGTDFTFTISSLQPEDIATYYCLQYDEFPYTFGGGTKVEIK

SEQ ID NO: 117 - protein, 107 aa, Artificial sequence
  Humanized antibody 38F8-Hu17/38F8-Hu27/38F8-Hu37 /38F8-Hu57/38F8-Hu67 light chain variable region
DIQMTQSPSSLSASVGDRVTITCQASQDISNYLTWFQQKPGKSPKTLIHRANRLVTGVPSRFSGSGSGTDYTFTISSLQPEDIAIYYCLQYDEFPYTFGGGTKVEIK

SEQ ID NO: 118 - protein, 107 aa, Artificial sequence
  Humanized antibody 38F8-Hu18/38F8-Hu28/38F8-Hu38/38F8-Hu58/38F8-Hu68 light chain variable region
DIQMTQSPSSLSASVGDRVTITCQASQDINSYLTWFQQKPGKSPKTLIHRANRLVTGVPSRFSGSGSGTDYTFTISSLQPEDIAIYYCLQYDEFPYTFGGGTKVEIK

SEQ ID NO: 119 - protein, 330 aa, Artificial sequence [sequence omitted]

SEQ ID NO: 120 - protein, 107 aa, Artificial sequence [sequence omitted]

SEQ ID NO: 121 - DNA, 363 bp, Artificial sequence
  Murine antibody 3D8.2.3 heavy chain variable region nucleotide sequence
gaagtgaagctggtggagtctgggggaggcttagtgaagcctggagggtccctgaaactctcctgtgcagcctctggattcactttcagtagctatgccatgtcttgggttcgccagactccagagaagaggctggagtgggtcgcatccattaatagtggtggtagcacctactatccagacagtgtgaagggccgattcaccatctccagagataatgccaggaacatcctgtacctgcaaatgagcagtctgaggtctgaggacacggccatgtattactgtgcaagagtgaattactacggctacggtgactatgctatggactactggggtcaaggaacctcagtcaccgtctcctca

SEQ ID NO: 122 - DNA, 321 bp, Artificial sequence
  Murine antibody 3D8.2.3 light chain variable region nucleotide sequence
gacatcaagatgacccagtctccatcttccatgtatgcgtctctaggagagagagtcactatcacttgcaaggcgagtcaggacattaatagctatttaagctggttccagcagaaaccagggaaatctcctaagaccctgatctatcgtgcaaacagattggtagatggggtcccatcaaggttcagtggcagtggatctgggcaagattattctctcaccatcagcagcctggagtatgaagatatgggaatttattattgtctacagtatgatgagtttccgtacacgttcggaggggggaccaacctggaaataaaa

SEQ ID NO: 123 - DNA, 354 bp, Artificial sequence
  Murine antibody 19F6.2.3 heavy chain variable region nucleotide sequence
gatgtacagcttcaggagtcaggacctggcctggtgaaaccttctcagtctctgtccctcacctgcactgtcactggctactcaatcaccagtgattatgcctggaactggatccggcagtttccaggaaacaaactggagtggatgggctacataagttacagtggtagcattaggtacaacccatctctcaaaagtcgaatctctatcactcgagacacatccaagaaccagttcttcctgcagttgaattctgtgactactgaggacacagccacatattactgtgcaagaggggagattacttattattttgactactggggccaaggcaccactctcacagtctcctca

SEQ ID NO: 124 - DNA, 321 bp, Artificial sequence
  Murine antibody 19F6.2.3 light chain variable region nucleotide sequence
gacatcaagatgacccagtctccagcatccctgtccatggctataggagaaaaagtcaccatcagatgcataaccaccactgatattgatgatgatatgaactggtaccagcagaagccaggggaacctcctaagctccttatttcagaaggcaatactcttcgtcctggagtcccatcccgattctccagcagtggctatggtacagattttgtttttacaattgaaaacatggtctcagaggatgttgcagattactactgtttgcaaagtaatgacttgccgctcacgttcggtgctgggaccaagctggagctgaaa

SEQ ID NO: 125 - DNA, 360 bp, Artificial sequence
  Murine antibody 38F8.1.1 heavy chain variable region nucleotide sequence
gaagtgaagctggtggagtctgggggagacttagtgaagcctggagggtccctgaaactctcctgtacagcctctggattcactttcagtaactatgccatgtcttgggttcgccagactccagagaagaggctggagtgggtcgcatccattagtagtggtggtcccacctactatccagacagtgtgaagggccgattcaccgtctccagagataatgccaggaacatcctgtacctgcaaatgagcagtctgaggtctgaagacacggccatgtattactgtgcaaggggctataggtacgacgtaaattggtacttcgatgtctggggcgcaggaacctcagtcaccgtctcctca

SEQ ID NO: 126 - DNA, 321 bp, Artificial sequence
  Murine antibody 38F8.1.1 light chain variable region nucleotide sequence
gacatcaagatgacccagtctccatcttccatgtatgcatctctaggagagagagtcactatcacttgcaaggcgagtcaggacattaatagctatttaacctggttccagcagaaaccagggaaatctcctaagaccctgatccatcgtgcaaacagattggtagatggggtcccatcaaggttcagtggcagtggatccgggcaagattattctctcaccatcagcagcctggaatatgaagatatgggaatttactattgtctacagtatgatgagtttccgtacacgttcggagggggggccaaggtggaaataaaa

SEQ ID NO: 127 - DNA, 354 bp, Artificial sequence
  Humanized antibody 19F6-Hu11/19F6-Hu12/19F6-Hu13/19F6-Hu14/19F6-Hu15 heavy chain variable region nucleotide sequence
caggttcagctgcaagagtctggccctggcctggtcaagcctagcgaaacactgagcctgacctgtaccgtgaccggctacagcatcaccagcgactacgcctggaactggatcagacagcctcctggcaaaggactggaatggatgggctacatcagctacagcggcagcatccggtacaagcccagcctgaaggaccggatcaccatcagcagagacaccagcaagaaccagttctccctgaagctgagcagcgtgacagccgccgatacagccgtgtactattgtgccagaggcgagatcacctactacttcgactattggggccagggcaccctggtcacagtctcttct

SEQ ID NO: 128 - DNA, 354 bp, Artificial sequence
  Humanized antibody 19F6-Hu21/19F6-Hu22/19F6-Hu23/19F6-Hu24/19F6-Hu25 heavy chain variable region nucleotide sequence
caggttcagctgcaagagtctggccctggcctggtcaagcctagcgaaacactgagcctgacctgtaccgtgtccggctacagcatcaccagcgactacgcctggaactggatcagacagcctcctggcaaaggactggaatggatgggctacatcagctacagcggcagcatccggtacaaccccagcctgaaggaccggatcaccatcagcagagacaccagcaagaaccagttctccctgaagctgagcagcgtgacagccgccgatacagccgtgtactattgtgccagaggcgagatcacctactacttcgactattggggccagggcaccctggtcacagtctcttct

SEQ ID NO: 129 - DNA, 354 bp, Artificial sequence; identical to SEQ ID NO: 128
  Humanized antibody 19F6-Hu31/19F6-Hu32/19F6-Hu33/19F6-Hu34/19F6-Hu35/19F6-Hu35V1/19F 6-Hu35V2/19F6-Hu35V3/19F6-Hu35V4/19F6-Hu35V5/19F6-Hu35V6/19F6-Hu3 5V7/19F6-Hu35V8/19F6-Hu35V9/19F6-Hu35V10 heavy chain variable

SEQ ID NO: 130 - DNA, 321 bp, Artificial sequence
  Humanized antibody 19F6-Hu11/19F6-Hu21/19F6-Hu31 light chain variable region nucleotide sequence
gacatccagatgacacagagccctagcagcctgtctgccagcgtgggagacagagtgaccatcacctgtatcaccaccaccgacatcgacgacgacatgaactggtatcagcagaagcccggcaaggcccctaagctgctgatctctgagggcaacacactgaggcctggcgtgccaagcagattttctggcagcggctacggcaccgacttcaccctgaccatatctagcctgcagcctgaggacttcgccacctactactgcctgcagagcaacgacctgcctctgacatttggccagggcaccaagctggaaatcaag

SEQ ID NO: 131 - DNA, 321 bp, Artificial sequence
  Humanized antibody 19F6-Hu12/19F6-Hu22/19F6-Hu32 light chain variable region nucleotide sequence
gacatccagatgacacagagccctagcagcctgtctgccagcgtgggagacagagtgaccatcacctgtatcaccaccaccgacatcgacgacgacatgaactggtatcagcagaagcccggcaaggcccctaagctgctgatctctgagggcaacacactgcagagcggcgtgccaagcagattttctggcagcggctacggcaccgacttcaccctgaccatatctagcctgcagcctgaggacttcgccacctactactgcctgcagagcaacgacctgcctctgacatttggccagggcaccaagctggaaatcaag

SEQ ID NO: 132 - DNA, 321 bp, Artificial sequence
  Humanized antibody 19F6-Hu13/19F6-Hu23/19F6-Hu33 light chain variable region nucleotide sequence
gacatccagatgacacagagccctagcagcctgtctgccagcgtgggagacagagtgaccatcacctgtagagccagcaccgacatcgacgacgacatgaactggtatcagcagaagcccggcaaggcccctaagctgctgatctacgagggcaacacactgcagagcggcgtgccaagcagattttctggcagcggctacggcaccgacttcaccctgaccatatctagcctgcagcctgaggacttcgccacctactactgcctgcagagcaacgacctgcctctgacatttggccagggcaccaagctggaaatcaag

SEQ ID NO: 133 - DNA, 321 bp, Artificial sequence
  Humanized antibody 19F6-Hu14/19F6-Hu24/19F6-Hu34 light chain variable region nucleotide sequence
gacatccagatgacacagagccctagcagcctgtctgccagcgtgggagacagagtgaccatcacctgtcagaccagcaccgacatcgacgacgacctgaactggtatcagcagaagcccggcaagcctcctaagctgctgatctccgagggcaacaccctggaaacaggcgtgccaagcagattttctggcagcggctctggcaccgacttcaccttcaccataagcagcctgcagcctgaggatatcgccgactactactgcctgcagagcaacgacctgcctctgacatttggagccggcaccaagctggaaatcaag

SEQ ID NO: 134 - DNA, 321 bp, Artificial sequence
  Humanized antibody 19F6-Hu15/19F6-Hu25/19F6-Hu35 light chain variable region nucleotide sequence
gagacaaccctgacacagagccctgccttcatgtctgccacacctggcgacaaagtgaccatcagctgcaaggccagcaccgacatcgacgacgacatgaactggtatcagcagaagcccggcgagcctcctaagctgatcatcagcgagggcaacacactgcggcctggcatccctcctagattttccagcagcggctacggcaccgacttcaccttcaccatcaacaacatcgagagcgaggacgccgccgactactactgcctgcagagcaatgatctgcccctgacctttggccagggcaccaagctggaaatcaag

SEQ ID NO: 135 - DNA, 321 bp, Artificial sequence
  Humanized antibody 19F6-Hu35V1 light chain variable region nucleotide sequence
gagacaaccctgacacagagccctgccttcatgtctgccacacctggcgacaaagtgaccatcagctgcaaggccagcaccagcatcgacgacgacatgaactggtatcagcagaagcccggcgagcctcctaagctgatcatcagcgagggcaacacactgcggcctggcatccctcctagattttccagcagcggctacggcaccgacttcaccttcaccatcaacaagatcaagagcgaggacgccgccacctactactgcctgcagagcaatgatctgcccctgacctttggccagggcaccaagctggaaatcaag

SEQ ID NO: 136 - DNA, 321 bp, Artificial sequence
  Humanized antibody 19F6-Hu35V2 light chain variable region nucleotide sequence
gagacaaccctgacacagagccctgccttcatgtctgccacacctggcgacaaagtgaccatcagctgcaaggccagcaccgacatcgacagcgacatgaactggtatcagcagaagcccggcgagcctcctaagctgatcatcagcgagggcaacacactgcggcctggcatccctcctagattttccagcagcggctacggcaccgacttcaccttcaccatcaacaagatcaagagcgaggacgccgccacctactactgcctgcagagcaatgatctgcccctgacctttggccagggcaccaagctggaaatcaag

SEQ ID NO: 137 - DNA, 321 bp, Artificial sequence
  Humanized antibody 19F6-Hu35V3 light chain variable region nucleotide sequence
gagacaaccctgacacagagccctgccttcatgtctgccacacctggcgacaaagtgaccatcagctgcaaggccagcaccagcatcgacgacgacatgaactggtatcagcagaagcccggcaagcctcctaagctgatcatcagcgagggcaacacactgcggcctggcatccctcctagattttccagcagcggctacggcaccgacttcaccttcaccatcaacaagatcgagagcgaggacgccgccacctactactgcctgcagagcaatgatctgcccctgacctttggccagggcaccaagctggaaatcaag

SEQ ID NO: 138 - DNA, 321 bp, Artificial sequence
  Humanized antibody 19F6-Hu35V4 light chain variable region nucleotide sequence
gagacaaccctgacacagagccctgccttcatgtctgccacacctggcgacaaagtgaccatcagctgcaaggccagcaccagcatcgacaacgacatgaactggtatcagcagaagcccggcaagcctcctaagctgatcatcagcgagggcaacacactgcggcctggcatccctcctagattttccagcagcggctacggcaccgacttcaccttcaccatcaacaagatcgagagcgaggacgccgccacctactactgcctgcagagcaatgatctgcccctgacctttggccagggcaccaagctggaaatcaag

SEQ ID NO: 139 - DNA, 321 bp, Artificial sequence
  Humanized antibody 19F6-Hu35V5 light chain variable region nucleotide sequence
gagacaaccctgacacagagccctgccttcatgtctgccacacctggcgacaaagtgaccatcagctgcaaggccagcaccgacatcgacgacgacatgaactggtatcagcagaagcccggcaagcctcctaagctgatcatcagcgagggcaacacactgcggcctggcatccctcctagattttccagcagcggctacggcaccgacttcaccttcaccatcaacaacatcaagagcgaggacgccgccacctactactgcctgcagagcaatgatctgcccctgacctttggccagggcaccaagctggaaatcaag

SEQ ID NO: 140 - DNA, 321 bp, Artificial sequence
  Humanized antibody 19F6-Hu35V6 light chain variable region nucleotide sequence
gagacaaccctgacacagagccctgccttcatgtctgccacacctggcgacaaagtgaccatcagctgcaaggccagcaccgacatcgacaacgacatgaactggtatcagcagaagcccggcaagcctcctaagctgatcatcagcgagggcaacacactgcggcctggcatccctcctagattttccagcagcggctacggcaccgacttcaccttcaccatcaacaacatcaagagcgaggacgccgccacctactactgcctgcagagcaatgatctgcccctgacctttggccagggcaccaagctggaaatcaag

SEQ ID NO: 141 - DNA, 321 bp, Artificial sequence
  Humanized antibody 19F6-Hu35V7 light chain variable region nucleotide sequence
gagacaaccctgacacagagccctgccttcatgtctgccacacctggcgacaaagtgaccatcagctgcaaggccagcaccagcatcgacgacgacatgaactggtatcagcagaagcccggcaagcctcctaagctgatcatcagcgagggcaacacactgcggcctggcatccctcctagattttccagcagcggctacggcaccgacttcaccttcaccatcaacaacatccagagcgaggacgccgccacctactactgcctgcagagcaatgatctgcccctgacctttggccagggcaccaagctggaaatcaag

SEQ ID NO: 142 - DNA, 321 bp, Artificial sequence
  Humanized antibody 19F6-Hu35V8 light chain variable region nucleotide sequence
gagacaaccctgacacagagccctgccttcatgtctgccacacctggcgacaaagtgaccatcagctgcaaggccagcaccgacatcgacaacgacatgaactggtatcagcagaagcccggcaagcctcctaagctgatcatcagcgagggcaacacactgcggcctggcatccctcctagattttccagcagcggctacggcaccgacttcaccttcaccatcaacaacatccagagcgaggacgccgccacctactactgcctgcagagcaatgatctgcccctgacctttggccagggcaccaagctggaaatcaag

SEQ ID NO: 143 - DNA, 321 bp, Artificial sequence
  Humanized antibody 19F6-Hu35V9 light chain variable region nucleotide sequence
gagacaaccctgacacagagccctgccttcatgtctgccacacctggcgacaaagtgaccatcagctgcaaggccagcaccagcatcgacgacgacatgaactggtatcagcagaagcccggcaagcctcctaagctgatcatcagcgagggcaacacactgcggcctggcatccctcctagattttccagcagcggctacggcaccgacttcaccttcaccatccggaagatcgagagcgaggacgccgccgattactactgcctgcagagcaacgatctgcccctgacatttggccagggcaccaagctggaaatcaag

SEQ ID NO: 144 - DNA, 321 bp, Artificial sequence
  Humanized antibody 19F6-Hu35V10 light chain variable region nucleotide sequence
gagacaaccctgacacagagccctgccttcatgtctgccacacctggcgacaaagtgaccatcagctgcaaggccagcaccgacatcgacagcgacatgaactggtatcagcagaagcccggcaagcctcctaagctgatcatcagcgagggcaacacactgcggcctggcatccctcctagattttccagcagcggctacggcaccgacttcaccttcaccatccggaagatcgagagcgaggacgccgccgattactactgcctgcagagcaacgatctgcccctgacatttggccagggcaccaagctggaaatcaag

SEQ ID NO: 145 - DNA, 363 bp, Artificial sequence
  Humanized antibody 3D8-HuC24/3D8-Hu25/3D8-Hu26 /3D8-Hu27 heavy chain variable region nucleotide sequence
gaggtgcagctggttgaatctggcggaggactggttcagcctggcggatctctgagactgtcttgtgccgccagcggcttcacctttagcagctacgccatgagctgggtccgacaggctcctggcaaaggccttgaatgggtcgccagcatcaatagcggcggcagcacctactatcccgacagcgtgaagggcagattcaccatcagccgggacaacgccaagaacagcctgtacctgcagatgaactccctgagagccgaggacaccgccgtgtactattgcgccagagtgaactactacggctacggcgattacgccatggactattggggccagggcaccctggttaccgttagctct

SEQ ID NO: 146 - DNA, 363 bp, Artificial sequence
  Humanized antibody 3D8-HuC44/3D8-Hu45/3D8-Hu46 /3D8-Hu47 heavy chain variable region nucleotide sequence
gaggtgcagctggttgaatctggcggaggactggttcagcctggcggatctctgagactgtcttgtgccgccagcggcttcacctttagcagctacgccatgagctgggtccgacaggctcctggcaaaggccttgaatgggtgtccagcatcaatagcggcggcagcacctactatcccgacagcgtgaagggcagattcaccatcagccgggacaacagcaagaacaccctgtacctgcagatgaacagcctgagagccgaggacaccgccgtgtactattgcgccagagtgaactactacggctacggcgattacgccatggactattggggccagggcaccctggttaccgttagctct

SEQ ID NO: 147 - DNA, 363 bp, Artificial sequence
  Humanized antibody 3D8-HuC 54/3D8-Hu55/3D8-Hu56 /3D8-Hu57 heavy chain variable region nucleotide sequence
gaggtgcagctggttgaatctggcggaggactggttcagcctggcggatctctgagactgtcttgtgccgccagcggcttcacctttagcagctacgccatgagctgggtccgacaggctcctggcaaaggccttgaatgggtgtccagcatcaatagcggcggcagcacctactatcccgacagcgtgaagggcagattcaccatcagcagagagaacgccaagaacagcctgtacctgcagatgaactccctgagagccggcgataccgccgtgtactattgcgccagagtgaactactacggctacggcgattacgccatggactattggggccagggcaccctggttaccgttagctct

SEQ ID NO: 148 - DNA, 363 bp, Artificial sequence
  Humanized antibody 3D8-HuC84/3D8-Hu85/3D8-Hu86 /3D8-Hu87 heavy chain variable region nucleotide sequence
gaggtgcagctggttgaatctggcggaggactggttcagcctggcggatctctgagactgtcttgtgccgccagcggcttcacctttagcagctacgccatgagctgggtccgacaggcccctgagaaaagactggaatgggtgtccagcatcagcagcggcggcagcacctactatcccgattctgtgaagggcagattcaccatcagccgggacaacagcaagaacaccctgtacctgcagatgaacagcctgagagccgaggacaccgccgtgtactattgcgccagagtgaactactacggctacggcgattacgccatggactattggggccagggcaccctggttaccgttagctct

SEQ ID NO: 149 - DNA, 363 bp, Artificial sequence
  Humanized antibody 3D8-HuC94/3D8-Hu95/3D8-Hu96 /3D8-Hu97 heavy chain variable region nucleotide sequence
gaggtgcagctggttgaatctggcggaggactggttcagcctggcggatctctgagactgtcttgtgccgccagcggcttcacctttagcagctacgccatgagctgggtccgacaggcccctgagaaaagactggaatgggtgtccagcatcagcaacggcggcagcacctactatcccgactctgtgaagggcagattcaccatcagccgggacaacagcaagaacaccctgtacctgcagatgaacagcctgagagccgaggacaccgccgtgtactattgcgccagagtgaactactacggctacggcgattacgccatggactattggggccagggcaccctggttaccgttagctct

SEQ ID NO: 150 - DNA, 321 bp, Artificial sequence
  Humanized antibody 3D8-HuC24/3D8-HuC44/3D8-HuC54 /3D8-HuC84/3D8-HuC94/38F8-Hu14/38F8-Hu24/38F8-Hu34/38F8-Hu54/38F8 -Hu64 light chain variable region nucleotide sequence
gagatcgtgatgacacagagccccgccacactgagtgtgtctccaggcgaaagagccacactgtcctgcaaggccagccaggacatcaacagctacctgagctggtatcagcagaagcccggacaggcccctaagctgctgatctacagagccaacagactggtggacggcatccccgccagattttctggctctggaagcggccaagagtacaccctgacaatcagcagcctgcagagcgaggacttcgccgtgtactactgcctgcagtacgacgagttcccctacacctttggcggaggcaccaaggtggaaatcaag

SEQ ID NO: 151 - DNA, 321 bp, Artificial sequence
  Humanized antibody 3D8-Hu25/3D8-Hu45/3D8-Hu55/3D8-Hu85/3D8-Hu95 light chain variable region nucleotide sequence
gacatccagatgacacagagccctagcagcctgtctgccagcgtgggagacagagtgaccattacctgtcaggccagccaggacatcaacagctacctgagctggttccagcagaagcctggcaaggcccctaagacactgatctaccgggccaacagactggtcacaggcgtgccaagcagattttctggcagcggctctggcaccgacttcaccttcaccataagcagcctgcagcctgaggatatcgccacctactactgcctgcagtacgacgagttcccctacacctttggcggaggcaccaagctggaaatcaag

SEQ ID NO: 152 - DNA, 321 bp, Artificial sequence
  Humanized antibody 3D8-Hu26/3D8-Hu46/3D8-Hu56/3D8-Hu86/3D8-Hu96 light chain variable region nucleotide sequence
gacatccagatgacacagagccctagcagcctgtctgccagcgtgggagacagagtgaccattacctgtcaggccagccaggacatcaacagctacctgagctggttccagcagaagcccggcaagagccccaagacactgatctacagagccaacagactggtcaccggcgtgcccagcagattttctggctctggcagcggcaccgactacaccttcaccatatctagcctgcagcctgaggatatcgccacctactactgcctgcagtacgacgagttcccttacacctttggcggaggcaccaagctggaaatcaag

SEQ ID NO: 153 - DNA, 321 bp, Artificial sequence
  Humanized antibody 3D8-Hu27/3D8-Hu47/3D8-Hu57/3D8-Hu87/3D8-Hu97 light chain variable region nucleotide sequence
gacatccagatgacacagagccctagcagcctgtctgccagcgtgggagacagagtgaccattacctgtcaggccagccaggacatcagcaactacctgagctggttccagcagaagcccggcaagagccccaagacactgatctacagagccaacagactggtcaccggcgtgcccagcagattttctggctctggcagcggcaccgactacaccttcaccatatctagcctgcagcctgaggatatcgccacctactactgcctgcagtacgacgagttcccttacacctttggcggaggcaccaagctggaaatcaag

SEQ ID NO: 154 - DNA, 360 bp, Artificial sequence
  Humanized antibody 38F8-Hu14/38F8-Hu16/38F8-Hu17 /38F8-Hu18 heavy chain variable region nucleotide sequence
gaggtgcagctggttgaatctggcggaggactggttcagcctggcggatctctgagactgagctgtaccgccagcggcttcaccttcagcaactacgccatgagctgggtccgacaggcccctggaaaaggccttgaatgggtcgccagcatctcttctggcggccctacctactacgccgactctgtgaagggcagattcaccgtgtccagagacaacagccggaacaccctgtacctgcagatgaacagcctgagagccgaggacaccgccgtgtactattgcgccagaggctacagatacgacgtgaactggtacttcgacgtgtggggcagaggcaccctggtcacagtttcttct

SEQ ID NO: 155 - DNA, 360 bp, Artificial sequence
  Humanized antibody 38F8-Hu24/38F8-Hu26/38F8-Hu27 /38F8-Hu28 heavy chain variable region nucleotide sequence
gaggtgcagctggttgaatctggcggaggactggttcagcctggcggatctctgagactgtcttgtgccgccagcggcttcaccttcagcaactacgccatgagctgggtccgacaggcccctggaaaaggccttgaatgggtcgccagcatctctagcggcggacccacctactatcccgactctgtgaagggcagattcaccgtgtccagagacaacagcaagaacaccctgtacctgcagatgaacagcctgagagccgaggacaccgccgtgtactattgcgccagaggctacagatacgacgtgaactggtacttcgacgtgtggggagccggcaccatggtcacagtttcttct

SEQ ID NO: 156 - DNA, 360 bp, Artificial sequence
  Humanized antibody 38F8-Hu34/38F8-Hu36/38F8-Hu37 /38F8-Hu38 heavy chain variable region nucleotide sequence
caggtgcagctggttgaatctggcggcggacttgtgaagcctggcggatctctgagactgagctgtgccgccagcggcttcaccttcagcaattacgccatgagctgggtccgacaggcccctggaaaaggccttgaatgggtcgccagcatctcttctggcggccctacctactacgccgactctgtgaagggcagattcaccatcagccgggacaacgccaagaacagcctgtacctgcagatgaactccctgagagccgaggacaccgccgtgtactattgcgccagaggctacagatacgacgtgaactggtacttcgacgtgtggggagccggcaccatggtcacagtttcttct

SEQ ID NO: 157 - DNA, 360 bp, Artificial sequence
  Humanized antibody 38F8-Hu54/38F8-Hu56/38F8-Hu57 /38F8-Hu58 heavy chain variable region nucleotide sequence
gaggtgcagctggttgaatctggcggaggactggttcagcctggcggatctctgagactgtcttgtgccgccagcggcttcaccttcagcaactacgccatgagctgggtccgacaggcccctgagaaaagactggaatgggtcgccagcatcagcagcggcggacctacctactatcccgactctgtgaagggcagattcaccgtgtccagagacaacagcaagaacaccctgtacctgcagatgaacagcctgagagccgaggacaccgccgtgtactattgcgccagaggctacagatacgacgtgaactggtacttcgacgtgtggggagccggcaccatggtcacagtttcttct

SEQ ID NO: 158 - DNA, 360 bp, Artificial sequence
  Humanized antibody 38F8-Hu64/38F8-Hu66/38F8-Hu67 /38F8-Hu68 heavy chain variable region nucleotide sequence
caggtgcagctggttgaatctggcggcggacttgtgaagcctggcggatctctgagactgagctgtgccgccagcggcttcaccttcagcaattacgccatgagctgggtccgacaggcccctgagaaaagactggaatgggtcgccagcatcagcagcggcggacctacctactatcccgactctgtgaagggcagattcaccatcagccgggacaacgccaagaacagcctgtacctgcagatgaactccctgagagccgaggacaccgccgtgtactattgcgccagaggctacagatacgacgtgaactggtacttcgacgtgtggggagccggcaccatggtcacagtttcttct

SEQ ID NO: 159 - DNA, 321 bp, Artificial sequence
  Humanized antibody 38F8-Hu16/38F8-Hu26/38F8-Hu36 /38F8-Hu56/38F8-Hu66 light chain variable region nucleotide sequence
gacatccagatgacacagagccctagcagcctgtctgccagcgtgggagacagagtgaccattacctgtcaggccagccaggacatcaacagctacctgacctggttccagcagaagcccggcaagagccccaagacactgatccacagagccaacagactggtcaccggcgtgccaagcagattttctggcagcggctctggcaccgacttcaccttcaccataagcagcctgcagcctgaggatatcgccacctactactgcctgcagtacgacgagttcccctacacctttggcggaggcaccaaggtggaaatcaag

SEQ ID NO: 160 - DNA, 321 bp, Artificial sequence
  Humanized antibody 38F8-Hu17/38F8-Hu27/38F8-Hu37 /38F8-Hu57/38F8-Hu67 light chain variable region nucleotide sequence
gacatccagatgacacagagccctagcagcctgtctgccagcgtgggagacagagtgaccattacctgtcaggccagccaggacatcagcaactacctgacctggttccagcagaagcccggcaagagccccaagacactgatccacagagccaacagactggtcaccggcgtgccaagcagattttctggcagcggctctggcaccgactacaccttcaccataagcagcctgcagcctgaggatatcgccatctactactgcctgcagtacgacgagttcccttacacctttggcggaggcaccaaggtggaaatcaag

SEQ ID NO: 161 - DNA, 321 bp, Artificial sequence
  Humanized antibody 38F8-Hu18/38F8-Hu28/38F8-Hu38/38F8-Hu58/38F8-Hu68 light chain variable region nucleotide sequence
gacatccagatgacacagagccctagcagcctgtctgccagcgtgggagacagagtgaccattacctgtcaggccagccaggacatcaacagctacctgacctggttccagcagaagcccggcaagagccccaagacactgatccacagagccaacagactggtcaccggcgtgccaagcagattttctggcagcggctctggcaccgactacaccttcaccataagcagcctgcagcctgaggatatcgccatctactactgcctgcagtacgacgagttcccttacacctttggcggaggcaccaaggtggaaatcaag